European Patent Specification EP 3 500 292 B1, published October 16, 2024. Title: SEA LICE VACCINE. Applicant: Pharmaq AS de la Fuente Garcia, Jose de Jesus Contreras Rojo, Marinela Villar Rayo, Margarita  Maria De Feijter Karlsen, Marius  Andre Brudeseth, Bjorn  Erik Lindmo Yttredal, Karine Wiik-Nielsen, Christer Ross Olsen, Rolf Hetlelid Hungerholdt, Liv Blom. The sequence listing filed with the application follows.

SEQUENCE LISTING (34 sequences)

SEQ ID NO: 1 - protein, 228 aa, Lepeophtheirus salmonis
MREEVPQRAIKADKLGFLARDANMVKMAKALEKGRSVSRDIGGSDPERMAPPRVEEYVRSVFKDSGVKIEVVAGHDTFEKEYPCLAAVNRAASTVARHQGRVIWLTYEPEGKVEKTAMIVGKGITYDTGGADIKAGGIMAGMSRDKCGAADAAGFMKTISELKPKNLKVVVGMAMVRNSVGSNCYVSDEIITSRAGVRIRVGNTDAEGRMAMVDVLCHMREKALREVN

SEQ ID NO: 2 - DNA, 684 bp, Lepeophtheirus salmonis
atgagggaagaggtgccacaaagggcgatcaaggcagataagttgggatttttggccagggacgctaatatggtgaagatggctaaggcattggagaaagggagatccgtatctagagacattggaggctctgatcctgaaagaatggcaccacctcgtgtggaggaatacgttcgttcagtctttaaggactctggtgttaaaattgaggttgttgcaggacacgacacctttgaaaaggagtatccgtgccttgctgctgtgaatcgtgcagcatccactgtagctcgtcatcaaggacgtgttatttggttgacatatgagcctgaaggaaaggtagaaaagacagccatgattgtaggaaagggtatcacttatgataccggtggagctgatatcaaggctggcggaatcatggctggaatgtccagggacaaatgtggagccgcagatgctgctggattcatgaaaaccatttcagaattgaagccaaagaacttgaaggtcgttgttggaatggctatggtgcggaatagtgttggatccaattgctatgtgtctgatgaaataattacctctcgtgctggagtaaggattcgtgtgggtaacacggatgctgagggtcgaatggccatggtagatgttctctgccacatgagagaaaaggctttaagagaagttaat

SEQ ID NO: 3 - protein, 191 aa, Lepeophtheirus salmonis
MAAIRKKLVIVGDGACGKTCLLIVFSKDQFPEVYVPTVFENYVADIEVDGKQVELALWDTAGQEDYDRLRPLSYPDTDVILMCFSIDSPDSLENIPEKWTPEVKHFCPNVPIILVGNKKDLRNDPNTIKELGKMKQEPVKPEDGRTMAEKINAFAYLECSAKSKEGVREVFETATRAALQVKKKKKRPCVL

SEQ ID NO: 4 - DNA, 573 bp, Lepeophtheirus salmonis
atggctgctattcgaaagaagttggtcattgttggggatggagcctgcggtaagacttgtctcctcatcgtcttcagtaaagatcagttcccagaagtctacgtcccaaccgtgtttgaaaactatgtggccgacatcgaagtggatggaaagcaggtggaactggcgctctgggatactgcaggccaagaagactatgatcgccttcgtcctttatcgtatccggacacggatgttattctcatgtgtttctctattgactctccggactcccttgagaacattccagagaaatggacgccggaagtcaaacatttttgccccaatgtacctataatactcgtggggaacaaaaaggatcttagaaatgacccaaacacgataaaagaattggggaaaatgaagcaagagccagtcaaacccgaagacggtcgcacaatggcggaaaaaatcaacgcatttgcttatttggaatgttccgctaaatctaaggaaggggtcagagaggtcttcgaaactgctacccgagccgcgttgcaagtgaagaaaaagaagaagagaccttgcgttcta

SEQ ID NO: 5 - protein, 58 aa, Lepeophtheirus salmonis
MADRNTEFELEELLQFKKSHEHEFSSATRTAEQAIEITKNNIAWMDSSYKTIQEWLNK

SEQ ID NO: 6 - DNA, 174 bp, Lepeophtheirus salmonis
atggctgacaggaatacggagtttgaacttgaagagctacttcaatttaaaaaatctcacgaacatgagtttagttcagcaactcgtaccgcagagcaagctattgaaataacgaagaataatatcgcctggatggactccagctataaaaccattcaagagtggttgaataaa

SEQ ID NO: 7 - protein, 67 aa, Lepeophtheirus salmonis
MMSMNGRLAFAIAAGAFGSSFQHGYNTGVLNAPQVLITNWLRGCEKNMTAVTEDGSDVLVCEKDMKS

SEQ ID NO: 8 - DNA, 201 bp, Lepeophtheirus salmonis
atgatgtccatgaatggaagattggcttttgctatagcagccggtgcatttggatcttcttttcaacatggatataataccggagttttgaatgctcctcaagttcttattacgaattggttgagaggatgtgagaaaaatatgacagcagttacagaggatggaagtgacgttcttgtctgtgagaaagatatgaaaagc

SEQ ID NO: 9 - protein, 72 aa, Lepeophtheirus salmonis
MYICDSEGNVICVDGWSYPSKLCSEPICDMNGRGCVNGKCIHPNVCACEVGWDGPNCDECIPLGGCKHGSCN

SEQ ID NO: 10 - DNA, 216 bp, Lepeophtheirus salmonis
atgtacatttgcgattcggaaggaaatgtcatctgtgttgatggatggtcttatccatctaaactctgtagtgaacctatctgtgatatgaatggaagaggatgcgttaatggaaaatgcatccatccaaatgtatgcgcatgtgaagttggatgggatggccctaactgtgatgaatgtattcctcttggtggttgtaagcatggaagctgtaac

SEQ ID NO: 11 - protein, 272 aa, Lepeophtheirus salmonis
MNEHVCSLFIYTDPFLWRHIYRSMKGSKRAERTRLKIEKLLTESVTRVNEAFSMAEFYGSGQTIHKGVHFSLLDYIIDDDTRCFSDTEYCDEKVMPMGEMCNEPIVCDNLKHVFCNNLTSLRFYLHAFSAFRNHGAFCLSYAFTYRNMSDFQGIAWVKGYDQSDERSLSHYGYCSLNDEKCQDESLQYYFRNTGVVNFHRLGENFSTSIGANVFIHEIGHSLGSTHDDKVSECNPQGHDLYLMTGKAENILLQRNSDRLSACSSREIGRNLD

SEQ ID NO: 12 - DNA, 816 bp, Lepeophtheirus salmonis
atgaatgaacatgtctgcagtttgttcatctacacagatccatttctctggagacacatttatcgctctatgaaaggaagtaaaagagcagaaaggacgaggctcaaaattgaaaaattactcacagaatccgtaacaagagtaaatgaggcattctctatggctgagttttatgggtctggtcagaccatacataagggagttcacttttccttactggattatatcatcgacgacgacacaagatgcttctcagacacggaatattgtgatgaaaaagtcatgcccatgggagaaatgtgcaatgagcccatcgtatgtgacaacttgaagcatgtcttttgtaacaacttaacaagtctacgtttctatctccatgctttttccgcatttcgcaaccatggagcattttgtctttcatatgcgtttacatataggaacatgagtgattttcaagggattgcatgggtaaagggatatgatcaaagcgatgagcgctctttgagtcactatggatattgctcattgaatgatgaaaagtgtcaggatgagagtctccaatattatttcaggaacacgggtgtagtcaattttcatagattaggagaaaatttttcaacgtcaattggagcaaatgtatttatacatgaaattggtcatagtttaggaagcacacacgacgataaagtgagtgagtgcaatccgcagggccatgacttgtatcttatgacgggaaaggctgagaacatattacttcagcgaaacagcgatcggctttctgcatgctcaagtcgggaaattggaaggaacttggat

SEQ ID NO: 13 - protein, 114 aa, Lepeophtheirus salmonis
MENSRADVPNIEDKIPPKIEEDNELQGNSLTVPKSSNRESSNVRRMHTAVRLNEVIVNKSHDAKLVILNLPSPPKIMGPDKDASYMEFLEVLTEGLERVLMVRGGGREVITIYS

SEQ ID NO: 14 - DNA, 342 bp, Lepeophtheirus salmonis
atggagaatagtcgagctgatgttccaaacattgaagacaaaataccacccaagattgaagaagataatgagttacaaggcaactctctcacagtaccaaagtcttcaaatcgtgagtcttctaacgtcagacggatgcatactgccgtacgattgaacgaagtgattgtcaacaagtcccacgatgcaaaattagtaattttgaatcttccaagtcctcccaaaattatgggtccagacaaagatgctagctatatggaatttttagaagttttaaccgagggtttagagcgagtccttatggttcgaggaggcggacgagaagtgattaccatttactct

SEQ ID NO: 15 - protein, 448 aa, Lepeophtheirus salmonis
MEFLGGFTINLAFITNGFALAYPTIALSQLTNNGTESCSFVMSKEEGSWFAGLLGIGGICGSVFFGTLIGQRIGNRKTLLLAAILDIIGWLLIAFAVNSPMMMGGRFLNGVFVGTIGPSGYTFLSEIMHRKHRASCSQATSVAISAGMLVTYGLGSVISWNLLAIGCGISSVLFFIMLLTMPDSPYWNASIGKIEEAKKSLSHFRSKKDDVEEEFKEIMEGIQKSIKKEKISFFEAMKLLFTDETCYKPFIILSVLFLIQTLSGLYAVIAYAIQVLEESRTPIDTNLGTIISGAMRLFFGTLAIPLFFYLPRKTLMYISTGLACLSISSLGILGLLELETNTFTTYFPVGAISLYMVSFTFGFQSIPFLYLGEYYPPHVRQHLAGLTSTLRFLGFFIMLKLFPQMMEFFGPNYTFIFLGLVCLFAGIYAKVVLPETKGLTLNQIQDLF

SEQ ID NO: 16 - DNA, 1344 bp, Lepeophtheirus salmonis
atggagtttttaggtggatttacgattaatcttgcatttattactaatggatttgccttggcctatcccacaattgcattgagtcaactcaccaataatggtactgaatcatgctcatttgttatgagcaaggaagagggatcctggttcgctggacttttgggcatcggaggtatttgtgggagtgtgttcttcggaactttgattggccaaagaattggtaatcgaaagactctcctcttggcagctattttagacattattggatggcttcttattgcatttgctgtgaattctccaatgatgatgggaggacgatttttaaatggtgtttttgttggcacaataggccctagtggatacaccttcctatcagaaataatgcatcgtaaacatcgagcttcttgttcacaagcaacttctgttgcaattagtgctgggatgctagtcacttatggactagggtctgtgatttcatggaacctccttgcgattggatgtggtatttcttcagttctgttctttatcatgttacttacaatgccagactctccatattggaatgcctctatcggaaaaattgaggaagccaagaaatctttaagtcatttcaggtcaaagaaggacgatgtggaagaagagttcaaagaaatcatggaaggaatacaaaaatccatcaaaaaagaaaagatttcattcttcgaggctatgaagttactcttcacggatgagacatgctacaaacctttcataatattaagcgttttgttcttaattcaaaccctttctgggttgtatgcagttattgcttatgctattcaagtattggaagagtccaggactcctattgatacaaatttgggcacaattatctccggagcaatgcgacttttttttggaactcttgcaattcccctcttcttttatctacctcgtaaaacactaatgtacatttccactggccttgcttgtctctctatttcctctctgggcattttgggtctcctagaattggaaacaaatacatttaccacatatttccccgttggtgcaatttctttatatatggtgtcatttacatttggattccagagcattcctttcctctatcttggagagtattatccacctcatgtgagacagcacttggcaggcttaacctccaccttaagattcttagggttttttatcatgctcaaattatttcctcaaatgatggagttctttggaccaaattatacatttatattcctaggacttgtatgtctctttgctggaatttacgccaaagtagttctccctgagacaaaggggcttactctgaatcaaattcaagacctattc

SEQ ID NO: 17 - protein, 542 aa, Lepeophtheirus salmonis
MYSGVQALTHLLEEVRVPYKVWILGEDSLDTLPWKEFALLLFQDFKTFVSINLFTRKLIFKYCSEYSVGIIVSATHQTPLPLKITNDSIFQRHNSLRNLFICPHSQIPNILKASRTLYETLDSYGFLSFTSRFLTKSTTPVLEAMSDSGPVTIVLHDRGQVPKIIFASNPLSHWLLKLLFLDSITFLSHQLINLDTKRWVLIDVDDIFVGKNRLSPSDVRELVISQDKLRKNIYGFKYNLGFSGYYFRNQGSSLINKEGDAALIEKKHHFWWFPHTFRHLQPHMFNSSLQLEQQMFLNKKFALEYKLPVNFHYAVAPHHSGVYPVHKPLYDAWKNVWGIVVTSTEEYPHLKPSRLRRGFTHDKLKILPRQTCGLFTKNIYYEDYPKNPEVLEKSIRGGELFQTISFNSINIFMTHMSNYGFDRLAPYTFESVFSMLKCWTNLKFVTVNPEKLSEIYFNMFPDEKVPIWGNPCYDSRLKEIWSKNKNCKRLPNFLVIGPQKTGTTALYNFLKIHPSIISNNHHSKYFEEVQFFSSSDYLKGFE

SEQ ID NO: 18 - DNA, 1626 bp, Lepeophtheirus salmonis
atgtactctggtgtccaagcattgactcacctcttggaagaagtccgtgttccctacaaagtgtggattttgggagaggactccttggacaccctaccttggaaggaattcgcccttcttctcttccaggattttaaaaccttcgtttctatcaacttgttcactcgaaaattgatatttaaatattgttcagaatattctgtcggtatcattgtatccgccacccatcaaacgcctcttcctttaaaaattaccaatgattccatttttcaacgtcataattcacttagaaatttatttatttgtcctcatagtcaaattcctaatattctaaaagcgtctcgtactctctatgaaactcttgactcttacgggttcttatcatttacttctcgttttctcactaaatctactacccctgtccttgaggcgatgtctgattccgggcctgttactatagttcttcatgatagaggacaagtaccaaagattatctttgcttcaaatcctttgagtcactggcttttaaagctacttttcctagactctattacttttttgagtcatcaacttattaacttagacactaaaaggtgggttctcatagatgttgacgatattttcgtcggcaaaaaccggctttctccatctgatgttagagagcttgttatctctcaagataaacttcgtaagaatatttatggatttaaatataacctgggattttctggctattatttccgtaaccaaggttcatctttaataaataaagaaggtgatgccgccctcattgaaaaaaaacaccatttttggtggttcccccatacattcagacatttacaacctcatatgttcaattcctcacttcaacttgaacagcagatgtttcttaataagaaatttgcgctggaatacaaattgccggtcaatttccattatgccgttgctccccatcattctggtgtttaccctgttcataagccattatatgatgcttggaaaaatgtctgggggatagttgttacttccacagaggaatatcctcaccttaaaccatctcgattacgtcgtggatttacacatgataaattaaaaattcttccgaggcaaacatgtggtctctttactaaaaacatttattatgaagattaccctaaaaatcctgaagtgttggaaaaatctatcagaggtggagaactgtttcagactatttcatttaattctataaatatattcatgacacatatgtccaattatggatttgatagactggctccgtatacttttgaatctgtattttccatgttaaaatgctggactaacctaaaatttgttacagttaatccggaaaagctaagtgaaatttattttaatatgtttcctgacgagaaagttccaatttggggaaatccttgttatgacagtcgccttaaagaaatctggtcgaaaaataaaaattgtaagaggctacctaattttcttgtgattggaccgcaaaaaactggaacaacggctttatataatttcctaaaaattcatccttcaataatttctaacaatcatcactccaaatattttgaagaagtacaatttttcagtagtagcgattatcttaaaggtttcgag

SEQ ID NO: 19 - protein, 282 aa, Lepeophtheirus salmonis
MEFYFGGNPIKCDCQMTWFKSINSVNGLQMFPTVADLESIYCELVYSREQSFVPLVEAESDNFLEYKAHCFALCQCCEYDACDCEMTCPSNCTCYHDNSWAKNIAECSFSNLKGLPDRLPMDATEIFLDGNEISVVQSHTFIGRKNLKILYLNESQVRYLPNNSFNGLIALEELHLENNHITRLEGSEFNGLFRLNKLYLHKNKISFVNNFTFKELKALETLYIHGNHISIFPPWVFFQNPLLATLTLSENPWNCDCNYMKRFENWIEGFHGKILDLYYVSC

SEQ ID NO: 20 - DNA, 849 bp, Lepeophtheirus salmonis
atggaattttactttggcggaaaccctattaaatgtgattgtcaaatgacatggttcaaaagtattaactcagttaatggtctacaaatgttccctactgttgctgatcttgagtcaatttattgtgaacttgtttattctcgtgaacagagttttgtgccacttgtggaagcagaaagtgacaattttctctgtgaatacaaggcacattgttttgctctatgccaatgttgtgaatatgatgcttgcgattgtgaaatgacttgcccttccaattgcacttgctaccatgacaattcttgggctaagaatattgctgaatgctcattttctaacctgaaaggacttcctgatcgtttgccaatggatgctacagaaatatttttagatggaaatgaaattagtgtagtgcagagtcatacgtttatcggtcggaagaaccttaagatattatacttgaatgaatctcaagtaagatatctgcccaataattcatttaatggattgatagcactcgaagaactacatttagaaaataatcatatcacaaggctggaaggaagtgaattcaacgggttgtttcgtctaaataaactttatttacacaaaaataagataagttttgtcaacaactttacatttaaagagttaaaagcattagagactctttatattcacggaaatcacatttccattttcccaccttgggtattttttcaaaatccattgctggctactcttactctctctgaaaacccatggaattgtgactgtaattatatgaaacgattcgaaaattggattgagggatttcatggtaaaatcttggatttgtactatgtatcttgt

SEQ ID NO: 21 - protein, 555 aa, Lepeophtheirus salmonis
MILIQSYVYLDAQNTAQHILYMDQASLGLLRINFVDSEKYKEIIKAYRTLQSSTAETLFKYLDINKPDDDKLNEDLESMFQFEKAIAGIMVPEDQRRNSTAMYNPMSLAKIMKSYTQIKWKIYFNELLKGDNAIEENDKIIVAEPYYFEKLNELLNETDDKIIYNYIHWRILLQTLPNGPDEMREHYKTFLKDAMGIKKEVLRDNICAKRVAAPFDGMGGLGFAVAYEYIQKKFDDDSKNEVKKMVGGLKSSFKELVAESSWMDKETQNKAKEKVDSMVQSLGYPDWLKTESEIEKKYKELDELKPKTLLENIKKVRQFESLTSFSAINSKPDKNAWPLHPAVVNAVYSPMRNSITFPAGILQYPFFESSNPMYLNFGSIGVVIGHEITHGFDDQGSQYDNNGNLVKWWSNSSLEAFQKEKECIIEQYSAFNVPEISEETYVNGVLTQGENIADNGGLRESFRAYKKWVNSNNDEPKLPELEKYTSEQMFFIAYSQTWCQVKTKASLQNQILSDPHSPGKFRSWGPVSNSKSFSKAFNCKPSDPMNNGENSCVLW

SEQ ID NO: 22 - DNA, 1665 bp, Lepeophtheirus salmonis
atgatcctgatccagagctacgtttacctggatgcgcagaacacggcgcagcacatcctgtacatggaccaagcgagcttagggctcctgagaattaactttgtggatagtgagaagtacaaagagataattaaggcgtaccgtaccctgcagagctccaccgcggaaaccctgttcaaatacttggatattaataaacctgacgatgacaaactgaacgaagatctggaatctatgttccagttcgaaaaagcaatcgctggcatcatggtgccggaagatcagcgtcgtaactctaccgcgatgtacaacccgatgtcgctggcgaaaatcatgaaatcttacacccagatcaaatggaaaatctacttcaacgaactgctgaaaggcgacaacgcaatcgaagaaaacgataaaatcatagtggcagaaccgtactacttcgaaaaactgaacgaactgctgaacgaaaccgacgacaaaattatctataactatatccactggcgtatcctgctgcagaccctgccgaacggcccggacgaaatgcgtgaacactacaaaaccttcctgaaagatgcgatgggtattaaaaaagaagttcttcgtgataacatctgcgcaaaacgcgttgccgctccgttcgacggcatgggtggtctgggcttcgcagttgcgtacgaatacattcagaaaaaattcgacgacgactccaaaaacgaagttaagaaaatggttggtggtctgaaaagcagcttcaaagaactggttgcggaaagctcctggatggataaagaaactcagaacaaagctaaagaaaaagtggattccatggttcagtccctgggttacccggactggctgaaaaccgaatctgaaatcgagaaaaaatataaagaactggatgaactgaaaccgaaaaccctgctggaaaacattaaaaaagttcgtcagttcgaaagcctgacttctttcagcgcgatcaacagcaaaccggataaaaacgcatggccgctgcacccggcggtggttaacgcggtttatagcccgatgcgtaactctattaccttcccggcgggcatcctgcagtacccgttcttcgaatctagcaacccgatgtacctgaacttcgggagcatcggcgtggttatcggccacgaaatcacccacggtttcgacgaccagggcagccagtacgataacaacggtaacctggtgaaatggtggtccaactccagcctggaagcctttcagaaagaaaaagaatgcatcatcgaacagtacagcgcgttcaacgttccggaaatctccgaagaaacctacgttaacggcgttctgacccagggcgaaaacatcgcggataacggcggcctgcgtgaatccttccgtgcgtataaaaaatgggtgaactccaacaacgacgaaccgaaactgccggaactggaaaaatacaccagcgaacagatgttcttcatcgcttactcccagacctggtgtcaggttaaaaccaaagcaagcctgcagaaccagatcctgagcgacccgcactctccgggcaaattccgcagctggggcccggtgtctaactctaaaagcttcagcaaagcgttcaactgcaaaccgagcgatccgatgaacaacggcgaaaacagctgcgtgctgtgg

SEQ ID NO: 23 - protein, 526 aa, Lepeophtheirus salmonis
MPMGVLACKSFSTSSKVGAAGGAEVSSILEERILGSAPKANLEETGRVLSIGDGIARVYGLKNIQAEEMVEFSSGLKGMALNLEADNVGVVVFGNDKLIKEGDVVKRTGAIVDVPVGRELLGRVVDALGNPIDGAGPVNTATRQRVGIKAPGIIPRQSVKEPMQTGIKAVDSLVPIGRGQRELIIGDRQTGKTAVAIDAIINQKRFNDAGDEKKKLYCIYVAIGQKRSTVAQIVKRLTDTDAMKYSIVVSATASDAAPLQYLAPYSGCAMGEFFRDNGMHALIIFDDLSKQAVAYRQMSLLLRRPPGREAYPGDVFYLHSRLLERAAKMSDTQGGGSLTALPVIETQAGDVSAYIPTNVISITDGQIFLETELFYKGIRPAINVGLSVSRVGSAAQTKSMKQVAGSMKLELAQYREVAAFAQFGSDLDAATQQLLNRGVRLTELLKQGQYVPMAIEDQVAVIYCGVRGFLDKLDPAKITDFEKKFLEHVRSSQKPLLDQIAKDGHLSDTSDKALHKVVVDFLATYQ

SEQ ID NO: 24 - DNA, 1578 bp, Lepeophtheirus salmonis
atgccgatgggcgttctggcgtgcaaatctttcagcacctcttctaaagttggcgcggcaggcggcgctgaagtttctagcatcctggaagaacgtatcctgggtagcgccccgaaagctaacctggaagaaaccggtcgcgttctgtctattggtgatggcattgcgcgcgtttatggcctgaaaaacatccaggcggaagaaatggttgaattcagcagcggtctgaaaggcatggcgctgaacctggaagctgataacgttggcgtggttgttttcggtaacgataaacttattaaagaaggtgatgttgttaaacgtaccggtgctatcgttgacgtgccggttggtcgtgaactgctgggccgtgttgtggatgccctgggaaacccaatcgatggcgcgggtccggtgaacaccgcgacccgccagcgcgtgggtatcaaagcgccgggtatcatcccgcgtcagtctgtaaaagaaccgatgcagaccggcattaaagcggttgactctctggttccgattggccgcggccagcgtgaactgatcattggcgaccgtcagactggcaaaaccgcggttgccatcgacgctatcatcaaccagaaacgtttcaacgatgcgggcgatgaaaagaaaaaactgtactgcatttacgttgctatcggtcagaaacgttctaccgttgcgcagatcgttaaacgtctgaccgacaccgacgcaatgaaatactctattgttgttagcgcgaccgccagcgatgctgcgccgctgcagtacctggctccgtacagcggctgtgctatgggggaattcttccgtgataacggtatgcatgctctgatcatcttcgatgatttatctaaacaggctgtagcctaccgtcagatgagcttgctgctgcgtcgcccgccgggccgtgaagcgtatccaggtgatgttttctacctgcactctcgcttgctggagcgtgctgcgaaaatgagcgacacccagggtggtggttccctgaccgcactgccggtgatcgaaacccaggcgggcgatgttagcgcttacatcccgaccaacgtgatcagcattaccgatggccagattttcctggaaaccgaactgttctacaaaggcatccgtccggccatcaacgtgggtctgtccgtgagccgcgttggttccgcggcacagaccaaatccatgaaacaggttgcgggtagcatgaaactggaactggcacagtaccgtgaagttgcagccttcgcgcagttcggctctgatctggacgctgcaacccagcagctgctgaaccgtggtgttcgtctgaccgaactgctgaaacagggccagtacgttccgatggcgattgaagatcaggttgctgtgatctactgcggcgttcgtggtttcctggacaaactggatccggcgaaaattaccgatttcgagaaaaaattcctggaacacgtgcgtagcagccagaaaccgctgctggaccagatcgctaaagatggccacctgagcgatacctccgataaagctctgcataaagttgttgttgacttcctggcgacctatcag

SEQ ID NO: 25 - protein, 515 aa, Lepeophtheirus salmonis
VELSVKCKDITNKDMMSKSDPICLVKQKTGVDKFEELGRTEQIKDCLSPEFMKKIVVPYNFEERQELRFELWDVDNIKKKVEDQKLLGYVDVSLGKIVNARGIEAKIEKGKGSMIIVAKEASSEQSSIGKLHLQFGASKLENKDTFGKSDPFFHISKSISATDFMKVYESEWIKNDLNPTWKPFSMSLNDLCDGELNRLLKIDVFDYSSNGKHDFIGEFETSVSQMMNKRSFEVINPKKKEKKKYTNSGVLNIISFNNDSPPSFLDFIQGGMVMNFSVAIDFTASNGNIRSRLSLHHRGDEGENDYTVAIQTVGDIIEDYDTDKKFPAFGFGARLPPNGEISHDFFLNLKENNPFCEGVRGILDAYYSTVDAVELYGPTNFSPCINRIKAIAQSHQDGKQYYVLLILTDGAITDMAETKKTIVEASNLPMSIIIIGVGSADFSSMIELDSDDALLKDEDGNVAARDIVQFVEMAKYVKKAENGDIFWDRASLAYQVMVEIPKQVLEWTSKRGIKP

SEQ ID NO: 26 - DNA, 1545 bp, Lepeophtheirus salmonis
gtggaactgagcgtcaaatgcaaagatatcaccaacaaagatatgatgtccaaaagcgatccgatctgcctggttaaacagaaaaccggcgttgacaaattcgaagaactgggccgtacggaacagatcaaagactgcctgagcccggaatttatgaagaaaatcgttgttccgtacaacttcgaagaacgccaggaactgcgcttcgaactgtgggatgtcgataacatcaagaaaaaagttgaagaccagaaactgctgggctatgttgatgttagcctgggcaaaatcgtgaacgcgcgtggaatcgaagcgaaaatcgaaaaaggtaaaggcagcatgatcatcgttgcgaaagaagcgtcctctgaacagagcagcatcggcaaactgcatctgcagttcggcgcgagcaaactggaaaacaaagatacctttggtaaatccgacccgttcttccatatctctaaaagcatcagcgcgaccgactttatgaaagtttacgaatccgaatggatcaaaaacgatctgaacccgacctggaaaccgttctctatgtcgctgaacgacctgtgcgacggcgaactgaaccgtctgctgaaaatcgacgttttcgattatagctctaacggcaaacacgacttcatcggcgaattcgaaaccagcgtgtcccagatgatgaacaaacggagcttcgaagttatcaacccgaagaaaaaagaaaagaaaaaatacaccaacagcggtgtgctgaacatcatcagctttaacaacgacagcccgccgtccttcctggatttcatccagggcggtatggttatgaacttcagcgttgccatcgatttcactgcgtctaacggtaacatccgttctcgtctgtccctgcaccatcgtggcgacgaaggtgaaaacgattacaccgtggccatccagaccgttggcgatatcattgaagactatgataccgataaaaaattcccggccttcggcttcggcgcgcgtctgccgccgaacggcgaaatcagccacgacttcttcctgaacctgaaagagaacaacccgttctgcgaaggtgtgcgtggcatcctggatgcgtactactctaccgtcgacgcggttgaactgtacggcccgaccaacttctccccgtgcatcaaccgtattaaagcgatcgcgcagagccaccaggatggcaaacagtactacgtcctgctgattctgaccgacggcgcgatcaccgacatggccgaaaccaaaaagaccatcgtggaagcgagcaacctgccgatgtctatcatcatcatcggcgtgggcagcgcggatttctcatctatgatcgaactggacagtgatgatgcattgttaaaagatgaggatggtaacgttgccgctcgtgatatcgttcagttcgttgaaatggccaaatacgtgaagaaagccgaaaacggtgacatcttctgggatcgcgcttctttagcgtaccaggtcatggtagaaatcccgaaacaggtgctggagtggacctctaaacgcggcattaaaccg

SEQ ID NO: 27 - protein, 567 aa, Lepeophtheirus salmonis
MPKAVNVRVTTIDAELEFAIQPNTTGKQLFDQVVKTIGLREIWFFGLQYTDTKGFSTWLKLNKKVMVQDVKKETPLQFKFRAKFYPEDVAEELIQDITLRLFYLQVKNAILSDEIYCPPETSVLLASYAVQSKHGDFQKDFHVAGFLANDRLLPERVTQQHRLNREQWEKRITEWYSEHKGMMREDAMMEYLKIAQDLEMYGVNYFEIKNKKGTELWLGVDALGLNIYEKDDRLTPKIGFPWSEIRNISFNDRKFVIKPIDAKAPNFVFFAPRLRINKRILTLCMGNHELYMRRRKPDTIEVQQMKAQNKEEKLAKQQEREKLQREIAAREKAERIQAEYEDRLKAMQEDMEKRQKALLEAQEQIKKLESVLRETQDAKQELEESQNELKDMMRRLEDDKNLEIEERTRLQDEIARKQSEVNDIYTQVQTKEQENMELQKEMDDARRKHEEATIALVAATTTPKHHHLEEDDNDDEVSNSERDLHVPSDPIDDPVSDRLLLVERNERLQNQLKSLKEDLSHTRDEGEETTMDRIHKENVKQGRDKYKTLREVRKGNTKRRVDQFENM

SEQ ID NO: 28 - DNA, 1701 bp, Lepeophtheirus salmonis
atgcctaaagcggtgaacgttagagtgacgaccattgacgctgagcttgagttcgcgatccagcctaacaccacaggtaaacagctgtttgatcaggtagtgaaaaccataggtctgcgtgaaatctggttcttcggcctgcagtacaccgataccaaaggtttctctacctggctgaaactgaacaaaaaagtgatggtgcaggatgttaaaaaagaaaccccgctgcagttcaaattccgtgcaaaattctacccggaagacgtggcggaagaactgatccaggacattaccctgcgtctgttctatctgcaggttaaaaacgcgattctgagtgatgagatctactgcccgcctgaaactagcgttctgttagctagctacgcggttcaatctaagcacggtgactttcaaaaagatttccatgttgcgggcttcctggcgaacgatcgcctgctgccggaacgtgttacccagcagcaccgtctgaaccgtgaacagtgggaaaaacgtatcaccgaatggtattccgaacataaaggcatgatgcgcgaagacgcgatgatggaatatctgaaaatcgcgcaggatctggaaatgtatggcgtgaactacttcgaaatcaagaacaaaaaaggcactgaactgtggctgggcgtggacgcactgggcctgaacatctacgaaaaagatgatcgcctgaccccgaaaatcggtttcccgtggagcgaaatccgtaacatcagcttcaacgaccgcaaattcgtcatcaaaccgattgatgctaaagcgccgaacttcgtgttcttcgctccgcgtctgcgcatcaacaaacgtatcctgaccctgtgtatgggcaaccacgaactgtacatgcgtcgtcgcaaaccggataccattgaagttcagcagatgaaagcacagaacaaagaagaaaaactggcgaaacagcaggaacgtgaaaaactgcagcgtgaaatcgcggcgcgtgaaaaagctgaacgcatccaggcggaatacgaagatcgtctgaaagcgatgcaggaagatatggaaaaacgtcagaaagcgctgctggaagcacaggaacagatcaaaaaactggaatccgttctgcgcgaaacccaggatgcgaaacaggaactggaagaatctcagaacgaactgaaagatatgatgcgtcgtctggaagacgacaaaaacctggaaatcgaagaacgtactcgcctgcaggacgaaatcgcccgcaaacagagcgaagttaacgatatctacacccaggtacagaccaaagaacaggaaaacatggaactgcagaaagaaatggatgacgcgcgtcgtaaacacgaagaagcgactatcgccctggttgcggcgaccaccaccccgaaacaccatcacctggaagaagatgataacgacgatgaagtttctaactctgaacgcgacctgcacgtgccgagcgacccgatcgacgacccggtttctgatcgtctgctgctggttgaacgtaacgaacgtctgcagaaccagctgaaatccctgaaagaagacctgagccacacccgtgacgaaggcgaagaaaccaccatggaccgtatccacaaagaaaacgttaaacagggtcgtgataaatacaaaaccctgcgtgaagttcgtaaaggtaacaccaaacgtcgtgttgatcagttcgaaaacatg

SEQ ID NO: 29 - protein, 206 aa, Lepeophtheirus salmonis
MNVPSSVSLVLILASTCHALMFHLEPNGRKCLKEEINKDILVSGEYEVTEVPGQVVDLIVVDSKGQHFVSRQNADKGKFAFTTDETNDAFEVCFISQIPAGHHGSQQEIFLSVKHGVEAKSYEGLGDAAKLKPLEVELKRLEDLSESIVQDFAHMRRREEEMRDTNESTNNRVLYFSIFSMCCLCSLATWQVLYLRKYFKSKKLIE

SEQ ID NO: 30 - DNA, 618 bp, Lepeophtheirus salmonis
atgaacgttccgagctctgtttctctggttctgatcctggcgagcacctgccacgcgctgatgttccacctggaaccgaacggtcgcaaatgcctcaaagaagaaatcaacaaagatatcctggtaagtggtgaatatgaagttacggaagtgcctggtcaggttgttgacctgatcgtagtcgactctaaaggtcagcactttgtttcccgccagaacgcagataaaggtaaattcgcgttcaccaccgatgaaaccaacgacgcgttcgaagtttgcttcatcagccagatcccggcgggtcaccacggctctcagcaggaaatcttcctgagtgttaaacatggtgttgaagcgaaaagctacgaaggactgggtgatgcggcgaaactgaaaccgctggaagttgagctgaaacgtctggaagatctgtcggaaagcatcgttcaggatttcgcgcacatgcgtcgtcgtgaagaagaaatgcgagataccaacgaatctaccaacaaccgtgttctgtacttcagcatcttcagcatgtgctgcctgtgctctctggcgacctggcaggttctgtacctgcgtaaatacttcaaatctaaaaaacttatcgaa

SEQ ID NO: 31 - protein, 711 aa, Lepeophtheirus salmonis
MVDEIQEKDKEIYELLSRIKSQDMELEKLNANFEQWKGIKNDLENKISILQRDLDEKYGVVQENNTVIDGLKIELQKLTEQKRECESFSNAEIQRIKETVEKLESENISIHQGIQEKDKAFALLEFQNKSLTQGNKQSIIHIDEMKALNTCLENKVKELQKNFELSSTRLDEANIKIAENEKEMNLVNTQLITVTDENQEWQHRFDELTNQNHSFAKEIEILKSSLDGENSKNNMDFKLLEGKNRELESFLEKAQLRIEDQGSNIHNLQLKLKSKNEKFINLENNIIFSNEQKLQLLSDVESYKNTSRSKEDDIKELQQLVDSLNNEKRDLTTRCDAYSTKKLQMESDFNECKNELRICELNTKELQSCVKSYEIELENVKFQLGECSRLQSILDEERKKFEVEKIKYQEDILTHSRSNNEEIAQFKIKCDKLESEMSKLKHDDSEFVELKSANSELLSKITCLSSQITLLLSEKEKIDEDLVRLTDSNEAVLQTKQHEIIELKEKINSILKDHKKEIEDTHNEYKEKMESSLYDGDSVKEEIASLQNLVKSKENDANLLNEQVNHKKEAITCLENRLSQEAVALSEVLNNNKKLVIEIEELKKLNCQLENNILEVSESQSKKEFDNLRQTLKSCKLELASTQVESTFKDKEIDTLRKDINFLSKKSNTYKEELRKVRNENMDTTIYNNESKLKKRNETKVERQNDAMHSV

SEQ ID NO: 32 - DNA, 2133 bp, Lepeophtheirus salmonis
atggttgacgaaatccaggaaaaagacaaagaaatctacgagctgctgtcccgtatcaaatcccaggacatggaactcgaaaaactgaacgcgaactttgaacagtggaaaggcatcaaaaacgacctggagaacaaaatctccattctgcagcgcgacctggatgaaaaatacggcgtggtgcaggagaacaacacggtgatcgacggcctgaaaatcgagctgcagaaactgaccgaacagaaacgtgaatgcgaaagcttcagcaacgcagagattcagcgtatcaaagaaaccgttgaaaagctggagtcggaaaacatcagcatccaccagggcatccaggagaaggacaaggccttcgctctcctggaattccagaacaaatccctgacgcagggtaacaaacagtccatcatccacatcgacgagatgaaggcgctgaacacctgccttgaaaacaaggttaaagaactgcagaaaaacttcgagctgagcagcacccgcctggatgaagccaacatcaagatcgcggagaacgagaaggagatgaacctggttaacacccagctgatcaccgttaccgacgagaaccaggagtggcagcaccgttttgacgaactgaccaaccagaaccacagcttcgctaaggagatcgagatcctgaaaagcagcctggacggcgaaaactccaagaacaacatggacttcaaactgctcgaaggcaaaaaccgcgaactggagagcttcctggaaaaggcgcagctgcgcatcgaagatcagggtagcaacatccacaacctgcagctgaaactgaagagcaaaaacgagaaattcatcaacctggaaaacaacattatcttctccaacgaacagaagctgcagctgctgtccgacgtggaatcctacaaaaacacctctcgcagcaaagaggatgatatcaaagaactgcagcagctcgtggactccctgaacaacgagaagcgcgacctgactacccggtgcgacgcgtacagcactaagaaactgcagatggagagcgacttcaacgaatgcaagaatgaactgcgcatctgcgaactgaacaccaaagagctgcagagctgcgtgaagtcctatgagatcgagctggagaacgtcaaattccagctgggcgaatgctcccgtctgcagtctatcctggatgaagaacgtaaaaaattcgaagttgaaaaaatcaaataccaggaagatatcctcactcactctcgcagcaacaacgaagaaatcgcacagttcaagatcaaatgcgataaactggaaagcgagatgtccaaactgaaacatgacgactctgaatttgtggaactcaaatccgcaaatagcgaactgctgtccaaaatcacctgtctcagcagccagattactctgctgctgagcgaaaaagaaaagatcgatgaagatctggtgcgcttgaccgatagcaacgaagccgtcctgcagacgaaacaacacgaaatcatcgaactgaaagaaaaaatcaactctatcctgaaagaccataaaaaagaaattgaagatacccacaacgaatataaagaaaaaatggaaagcagcctgtacgacggtgattccgttaaagaagagatcgcctccctgcagaacctggttaaatctaaggaaaacgacgcaaacctgctgaacgagcaggttaaccacaagaaagaagcgattacctgcctggaaaaccgtctgtcccaggaagcagttgcgctgagcgaagtgctgaacaacaacaaaaaactggttatcgaaatcgaagaactgaaaaaactgaattgccagctggaaaacaacattcttgaggtttctgaatcccagtctaaaaaagaattcgacaacttgcgccagactctgaaaagctgcaaactggaactggcttccactcaggtagagtctactttcaaagataaagaaattgataccctgcgtaaagatattaacttcctgtctaaaaaatctaacacctacaaagaagaactgcgtaaagttcgtaacgaaaacatggacaccaccatctataacaacgaatctaaactgaaaaaacgtaatgagactaaagttgaacgtcagaacgacgcgatgcatagcgtg

SEQ ID NO: 33 - protein, 308 aa, Lepeophtheirus salmonis
MSTEDKEGLESIRMLHSHLDDDKDGSIEPAETGEFIRGGELRGEDYIKRQKLFHRSDVEITVLDLWQTWTTSTVHNWTVDQTIEWLLTSVDLPQYKTTFEYHSVNGSRIPQIAVNSSYLTKVLKITNPIHKSKLSLKAMDVVLFGPPKEPSSFFKDVIFTIIILLAGTGLFYAYHKNKKSQDQLKKMMEDMDKLGVAERDLLDLQSKLQQKDKVIKNIRSVSKELNQVSLETEEIKRMREEIEDLRNQLYAAETELEDKCWSAPPTLQLWLQISYEIESMGFSAKKKEAEKQLELAKDMCEKLKKKRS

SEQ ID NO: 34 - DNA, 924 bp, Lepeophtheirus salmonis
atgagcactgaagataaagaaggcctggagagcatccgtatgctgcacagccacctggatgatgataaagatggtagcatcgaaccggcggaaaccggtgaattcatccgtggtggcgaactgcgtggcgaagactacatcaaacgccagaaactgttccaccgtagcgatgttgaaatcaccgtgctggatctgtggcagacctggaccaccagcaccgtgcacaactggaccgtggatcagaccatcgagtggctgctgaccagcgtggacctgccgcagtacaaaaccaccttcgaataccactctgttaacggcagccgcatcccgcagatcgcggttaacagcagctacctgaccaaagttctgaaaattaccaacccgatccacaaaagcaaactgagcctgaaagcgatggacgttgtgctgttcggtccgccgaaagaaccgagctctttcttcaaagatgttatcttcaccatcatcatcctgctggccggcaccggtctgttctacgcttaccacaaaaacaaaaaatcccaggaccagctgaaaaagatgatggaagatatggataaactgggcgttgcggaacgtgacctgctggatctgcagtctaaactgcaacagaaagacaaagtcatcaaaaacattcgtagcgttagcaaagaactgaaccaggtttctctggaaaccgaagaaatcaaacgtatgcgtgaagaaatcgaagatctgcgtaaccagctgtacgcggcggaaaccgaactggaagacaaatgctggtccgccccaccgaccttgcagctgtggctgcagatttcatacgaaatcgaatccatgggcttttcagcgaaaaagaaagaagctgagaaacagctggaactcgctaaagatatgtgcgagaaactcaaaaagaaacgctct